European Patent Application EP 4 420 670 A1, published August 28, 2024. Title: NON-COVALENT BINDING PEPTIDE AND CARRIER COMPLEX COMPRISING IT. Applicant: Consejo Superior de Investigaciones Cientificas (CSIC). The sequence listing filed with the application follows.

SEQUENCE LISTING (15 sequences)

SEQ ID NO: 1 - protein, 182 aa, synthetic construct
  source 1..182: note = peptide P40N1 fragment of the bacterial protein P40; note (original language) = peptido P40N1 fragmento de la proteina bacteriana P40; organism (original language) = construccion sintetica
DTSDSIASNKSETNALLKQIEDANTEVINLNKQIDTKNGQISDATAKISATDAKISSLSGEIVAAQKNVTARKNNLKDQLISLQKKAGNSVSGNVYIDFVLNSQNLSDLIARTMTVGKLSQASKDALDAVTVAKDKLAGLKTEQENARQTLVSTKASLETQKSQLVSLQKDANDKQDALNKQ

SEQ ID NO: 2 - protein, 271 aa, synthetic construct
  source 1..271: note = peptide P40N2 fragment of the bacterial protein P40; note (original language) = peptido P40N2 fragmento de la proteina bacteriana P40; organism (original language) = construccion sintetica
DTSDSIASNKSETNALLKQIEDANTEVINLNKQIDTKNGQISDATAKISATDAKISSLSGEIVAAQKNVTARKNNLKDQLISLQKKAGNSVSGNVYIDFVLNSQNLSDLIARTMTVGKLSQASKDALDAVTVAKDKLAGLKTEQENARQTLVSTKASLETQKSQLVSLQKDANDKQDALNKQIADHKDELVALQSQFAQEQSEAAAATQAALKTVAASTASSSTTSSSSSATSTSTIANNTSSSSNNSSSIINNNTTSGSGSHADYSSSGN

SEQ ID NO: 3 - protein, 411 aa, Lacticaseibacillus paracasei
  source 1..411: note = Bacterial protein P40; note (original language) = Proteina bacteriana P40
MKFNKVMITLVAAVTLAGSASAVTPVFADTSDSIASNKSETNALLKQIEDANTEVINLNKQIDTKNGQISDATAKISATDAKISSLSGEIVAAQKNVTARKNNLKDQLISLQKKAGNSVSGNVYIDFVLNSQNLSDLIARTMTVGKLSQASKDALDAVTVAKDKLAGLKTEQENARQTLVSTKASLETQKSQLVSLQKDANDKQDALNKQIADHKDELVALQSQFAQEQSEAAAATQAALKTVAASTASSSTTSSSSSATSTSTIANNTSSSSNNSSSIINNNTTSGSGSHADYSSSGNTYPWGQCTWYVKSVASWAGNGWGNGAQWGSSAAAAGFTVNHTPAAGSIIVFAAGQSVGGQWTADGSYGHVAYVQSVSGDSVTISQGGMGFSSPTGPNTQTISGASSYVYIHR

SEQ ID NO: 4 - protein, 7 aa, synthetic construct
  source 1..7: note = targeting peptide; note (original language) = peptido de direccionamiento; organism (original language) = construccion sintetica
LQNAPRS

SEQ ID NO: 5 - protein, 7 aa, synthetic construct
  source 1..7: note = targeting peptide; note (original language) = peptido de direccinamiento; organism (original language) = construccion sintetica
APSPMIW

SEQ ID NO: 6 - protein, 7 aa, synthetic construct
  source 1..7: note = targeting peptide; note (original language) = peptido de direccionamiento; organism (original language) = construccion sintetica
QMAQWPP

SEQ ID NO: 7 - protein, 7 aa, synthetic construct
  source 1..7: note = targeting peptide; note (original language) = peptido de direccionamiento; organism (original language) = construccion sintetica
APLPRPG

SEQ ID NO: 8 - protein, 7 aa, synthetic construct
  source 1..7: note = targeting peptide; note (original language) = peptido de direccionamiento; organism (original language) = construccion sintetica
ATWLPPR

SEQ ID NO: 9 - protein, 189 aa, synthetic construct
  source 1..189: note = Fusion P40N1-LQN, fusion of peptides of sequences SEQ ID NO:1 and SEQ ID NO: 4; note (original language) = Fusion P40N1-LQN, fusion de los peptideos de secuencia SEQ ID NO: 1 y SEQ ID NO: 4; organism (original language) = construccion sintetica
DTSDSIASNKSETNALLKQIEDANTEVINLNKQIDTKNGQISDATAKISATDAKISSLSGEIVAAQKNVTARKNNLKDQLISLQKKAGNSVSGNVYIDFVLNSQNLSDLIARTMTVGKLSQASKDALDAVTVAKDKLAGLKTEQENARQTLVSTKASLETQKSQLVSLQKDANDKQDALNKQLQNAPRS

SEQ ID NO: 10 - protein, 189 aa, synthetic construct
  source 1..189: note = Fusion P40N1-APS, fusion of peptides of sequences SEQ ID NO:1 and SEQ ID NO:5; note (original language) = Fusion P40N1-APS, usion de los peptidos de secuenia SEQ ID NO:1 y SEQ ID NO:5; organism (original language) = construccion sintetica
DTSDSIASNKSETNALLKQIEDANTEVINLNKQIDTKNGQISDATAKISATDAKISSLSGEIVAAQKNVTARKNNLKDQLISLQKKAGNSVSGNVYIDFVLNSQNLSDLIARTMTVGKLSQASKDALDAVTVAKDKLAGLKTEQENARQTLVSTKASLETQKSQLVSLQKDANDKQDALNKQAPSPMIW

SEQ ID NO: 11 - DNA, 23 bp, synthetic construct
  source 1..23: mol_type = other DNA; note = Primer forward LCP40N_for; note (original language) = Cebador directo LCNP40N_for; organism (original language) = construccion sintetica
gttggatccgatacaagcgacag

SEQ ID NO: 12 - DNA, 27 bp, synthetic construct
  source 1..27: mol_type = other DNA; note = Primer reverse (rev) LcaP40N1-rev; note (original language) = Cebador reverso LcaP40N1-rev; organism (original language) = construccion sintetica
gtagggcccttattgcttattcaaagc

SEQ ID NO: 13 - DNA, 26 bp, synthetic construct
  source 1..26: mol_type = other DNA; note = Primer reverse LCP40N2-rev; note (original language) = Cebador reverso LCP40N2-rev; organism (original language) = construccion sintetica
gttggtaccttagttgcctgaactgc

SEQ ID NO: 14 - DNA, 44 bp, synthetic construct
  source 1..44: mol_type = other DNA; note = CD133_cancer recognizing peptide APSPMIW primer Fw_v2; note (original language) = Cebador directo peptido APSPMIW de reconocimiento de CD133; organism (original language) = construccion sintetica
gctccgtctccgatgatctggtaaccttaattagctgagcttgg

SEQ ID NO: 15 - DNA, 44 bp, synthetic construct
  source 1..44: mol_type = other DNA; note = CD133_ cancer recognizing peptide LQNAPRS primer Fw_v2; note (original language) = Cebador directo peptido LQNAPRS de reconocimiento de CD133; organism (original language) = construccion sintetica
ctgcagaacgctccgcgttcttaaccttaattagctgagcttgg